European Patent Specification EP 3 666 791 B1, published June 19, 2024. Title: MODIFIED FIBROBLAST GROWTH FACTORS-1 FOR THE TREATMENT OF OCULAR DISORDERS. Applicant: Trefoil Therapeutics LLC. The sequence listing filed with the application follows.

SEQUENCE LISTING (4 sequences)

SEQ ID NO: 1 - protein, 140 aa, Homo Sapiens
FNLPPGNYKKPKLLYCSNGGHFLRILPDGTVDGTRDRSDQHIQLQLSAESVGEVYIKSTETGQYLAMDTDGLLYGSQTPNEECLFLERLEENHYNTYISKKHAEKNWFVGLKKNGSCKRGPRTHYGQKAILFLPLPVSSD

SEQ ID NO: 2 - protein, 140 aa, Homo Sapiens
FNLPPGNYKKPVLLYCSNGGHFLRILPDGTVDGTRDRSDQHIQLQLSAESVGEVYIKSTETGQYLAMDTDGLLYGSQTPNEECLFLERLEENHYNTYISKKHAEKNWFVGLKKNGSVKRGPRTHYGQKAILFLVLPVSSD

SEQ ID NO: 3 - protein, 140 aa, Homo Sapiens
FNLPPGNYKKPKLLYSSNGGHFLRILPDGTVDGTRDRSDQHIQLQLSAESVGEVYIKSTETGQYLCMDTDGLLYGSQTPNEECLFLERLEENHYNTYISKKHAEKNWFVGLKKNGSVKRGPRTHYGQKAILFLPLPVSSD

SEQ ID NO: 4 - protein, 140 aa, Homo Sapiens
FNLPPGNYKKPVLLYSSNGGHFLRILPDGTVDGTRDRSDQHIQLQLSAESVGEVYIKSTETGQYLCMDTDGLLYGSQTPNEECLFLERLEENHYNTYISKKHAEKNWFVGLKKNGSVKRGPRTHYGQKAILFLVLPVSSD